European Patent Application EP 4 653 549 A1, published November 26, 2025. Title: PROBE METHOD-BASED KIT AND METHOD FOR TRACKING BEHAVIOR TRAJECTORY OF ACIPENSER DABRYANUS DUMERIL RELEASED UPSTREAM OF YANGTZE RIVER. Applicant: CHINESE STURGEON RESEARCH INSTITUTE, CHINA THREE GORGES CORPORATION. Application CN. The sequence listing filed with the application follows.

SEQUENCE LISTING (3 sequences)

SEQ ID NO: 1 - DNA, 19 bp, synthetic construct
  source 1..19: mol_type = other DNA
ggtcgccctgacaacttgc

SEQ ID NO: 2 - DNA, 20 bp, synthetic construct
  source 1..20: mol_type = other DNA
agtgagggggagcatggtgt

SEQ ID NO: 3 - DNA, 26 bp, synthetic construct
  source 1..26: mol_type = other DNA
acatccagccaactaggcctaatgat